European Patent Specification EP 3 609 542 B1, published February 22, 2023. Title: Adeno-Associated Virus Library. Applicant: Ruprecht-Karls-Universität Heidelberg. The sequence listing filed with the application follows.

SEQUENCE LISTING (52 sequences)

SEQ ID NO: 1 - protein, 4 aa, Artificial
  generic recognition motif, X = any amino acid
  misc_feature (2)..(3): Xaa can be any naturally occurring amino acid
NXXR

SEQ ID NO: 2 - protein, 7 aa, Artificial
  generic recognition motif, X = any amino acid
  misc_feature (2)..(3): Xaa can be any naturally occurring amino acid
  misc_feature (5)..(7): Xaa can be any naturally occurring amino acid
NXXRXXX

SEQ ID NO: 3 - protein, 9 aa, Artificial
  inserted binding peptide
CDCRGDCFC

SEQ ID NO: 4 - protein, 7 aa, Artificial
  inserted binding peptide
NDVRSAN

SEQ ID NO: 5 - protein, 7 aa, Artificial
  inserted binding peptide
NDVRAVS

SEQ ID NO: 6 - protein, 7 aa, Artificial
  inserted binding peptide
MPLGAAG

SEQ ID NO: 7 - protein, 7 aa, Artificial
  inserted binding peptide
NYSRGVD

SEQ ID NO: 8 - protein, 7 aa, Artificial
  inserted binding peptide
NEARVRE

SEQ ID NO: 9 - protein, 11 aa, Artificial
  binding peptide
GCDCRGDCFCA

SEQ ID NO: 10 - protein, 9 aa, Artificial
  binding peptide
GNDVRSANA

SEQ ID NO: 11 - protein, 9 aa, Artificial
  binding peptide
GNDVRAVSA

SEQ ID NO: 12 - protein, 9 aa, Artificial
  binding peptide
GMPLGAAGA

SEQ ID NO: 13 - protein, 9 aa, Artificial
  binding peptide
GNYSRGVDA

SEQ ID NO: 14 - protein, 9 aa, Artificial
  binding peptide
GNEARVREA

SEQ ID NO: 15 - protein, 6 aa, Artificial
  Variant 1 insertion site AAV1 and AAV6
  MISC_FEATURE (3)..(4): insertion site
STDPAT

SEQ ID NO: 16 - protein, 6 aa, Artificial
  Variant 1 insertion site AAV2
  MISC_FEATURE (3)..(4): insertion site
GNRQAA

SEQ ID NO: 17 - protein, 6 aa, Artificial
  Variant 1 insertion site AAV3b
  MISC_FEATURE (3)..(4): insertion site
LQSSNT

SEQ ID NO: 18 - protein, 6 aa, Artificial
  Variant 1 insertion site AAV4
  MISC_FEATURE (3)..(4): insertion site
DQSNSN

SEQ ID NO: 19 - protein, 6 aa, Artificial
  Variant 1 insertion site AAV5
  MISC_FEATURE (3)..(4): insertion site
NQSSTT

SEQ ID NO: 20 - protein, 6 aa, Artificial
  Variant 1 insertion site AAV7
  MISC_FEATURE (3)..(4): insertion site
AANTAA

SEQ ID NO: 21 - protein, 6 aa, Artificial
  Variant 1 insertion site AAV8
  MISC_FEATURE (3)..(4): insertion site
QQNTAP

SEQ ID NO: 22 - protein, 6 aa, Artificial
  Variant 1 insertion site AAV9
  MISC_FEATURE (3)..(4): insertion site
SAQAQA

SEQ ID NO: 23 - protein, 6 aa, Artificial
  Variant 1 insertion site AAVrh10
  MISC_FEATURE (3)..(4): insertion site
QQNAAP

SEQ ID NO: 24 - protein, 6 aa, Artificial
  Variant 1 insertion site AAVpo.1
  MISC_FEATURE (3)..(4): insertion site
NQNSNT

SEQ ID NO: 25 - protein, 6 aa, Artificial
  Variant 1 insertion site AAV12
  MISC_FEATURE (3)..(4): insertion site
NQNATT

SEQ ID NO: 26 - protein, 6 aa, Artificial
  Variant 2 insertion site AAV1 and AAV6
  MISC_FEATURE (3)..(4): insertion site
SSSTDP

SEQ ID NO: 27 - protein, 6 aa, Artificial
  Variant 2 insertion site AAV2
  MISC_FEATURE (3)..(4): insertion site
RGNRQA

SEQ ID NO: 28 - protein, 6 aa, Artificial
  Variant 2 insertion site AAV3b
  MISC_FEATURE (3)..(4): insertion site
SSNTAP

SEQ ID NO: 29 - protein, 6 aa, Artificial
  Variant 2 insertion site AAV4
  MISC_FEATURE (3)..(4): insertion site
SNSNLP

SEQ ID NO: 30 - protein, 6 aa, Artificial
  Variant 2 insertion site AAV5
  MISC_FEATURE (3)..(4): insertion site
SSTTAP

SEQ ID NO: 31 - protein, 6 aa, Artificial
  Variant 2 insertion site AAVpo.1
  MISC_FEATURE (3)..(4): insertion site
NSNTHP

SEQ ID NO: 32 - protein, 6 aa, Artificial
  Variant 2 insertion site AAV12
  MISC_FEATURE (3)..(4): insertion site
NATTAP

SEQ ID NO: 33 - protein, 11 aa, Artificial
  AAV2 wt insertion site
  MISC_FEATURE (5)..(6): insertion site
TNLQRGNRQAA

SEQ ID NO: 34 - DNA, 33 bp, Artificial
  AAV2 wt insertion site encoding
accaacctccagagaggcaacagacaagcagct

SEQ ID NO: 35 - protein, 12 aa, Artificial
  AAV2 NIS
  MISC_FEATURE (7)..(8): insertion site
TNLQGQRGAQAA

SEQ ID NO: 36 - DNA, 36 bp, Artificial
  AAV2 NIS encoding
accaacctccagggccagagaggcgcccaggcggcc

SEQ ID NO: 37 - protein, 13 aa, Artificial
  AAV2 2xA
  MISC_FEATURE (10)..(11): insertion site
TNLQRGNAAAAAR

SEQ ID NO: 38 - DNA, 39 bp, Artificial
  AAV2 2xA encoding
accaacctccagagaggcaacgcggcggcagcagccaga

SEQ ID NO: 39 - protein, 14 aa, Artificial
  AAV2 3xA
  MISC_FEATURE (10)..(11): insertion site
TNLQRGNAAAAAAR

SEQ ID NO: 40 - DNA, 42 bp, Artificial
  AAV2 3xA encoding
accaacctccagagaggcaacgcggcggcagcagccgcgaga

SEQ ID NO: 41 - protein, 15 aa, Artificial
  AAV2 4xA
  MISC_FEATURE (10)..(11): insertion site
TNLQRGNAAAAAAAR

SEQ ID NO: 42 - DNA, 45 bp, Artificial
  AAV2 4xA encoding
accaacctccagagaggcaacgcggcggcagcagccgcggccaga

SEQ ID NO: 43 - protein, 16 aa, Artificial
  AAV2 wt extended
TNLQRGNRQAATADVN

SEQ ID NO: 44 - protein, 25 aa, Artificial
  AAV2_A2(OIS)
TNLQRGQRGNYSRGVDAQAATADVN

SEQ ID NO: 45 - protein, 25 aa, Artificial
  AAV2_A2(NIS)
TNLQGQRGNYSRGVDAQAAATADVN

SEQ ID NO: 46 - protein, 28 aa, Artificial
  AAV2_A2_2xA(NIS)
TNLQRGNAAANYSRGVDAARQAATADVN

SEQ ID NO: 47 - protein, 29 aa, Artificial
  AAV2_A2_3xA(NIS)
TNLQRGNAAANYSRGVDAAARQAATADVN

SEQ ID NO: 48 - protein, 30 aa, Artificial
  AAV2_A2_4xA(NIS)
TNLQRGNAAANYSRGVDAAAARQAATADVN

SEQ ID NO: 49 - protein, 7 aa, Artificial
  inserted binding peptide
NSSRDLG

SEQ ID NO: 50 - protein, 7 aa, Artificial
  inserted binding peptide
SEGLKNL

SEQ ID NO: 51 - protein, 7 aa, Artificial
  inserted binding peptide
PSVPRPP

SEQ ID NO: 52 - protein, 7 aa, Artificial
  inserted binding peptide
NFTRLSA